European Patent Application EP 4 358 097 A1, published April 24, 2024. Title: METHODS OF DETERMINING TISSUES AND/OR CELL TYPES GIVING RISE TO CELL-FREE DNA, AND METHODS OF IDENTIFYING A DISEASE OR DISORDER USING SAME. Applicant: University of Washington. Application WO PCT/US2015/042310, filed July 27, 2015. The sequence listing filed with the application follows.

SEQUENCE LISTING (4 sequences)

SEQ ID NO: 1 - DNA, 34 bp, synthetic construct
  misc_feature 1..34: note = Synthetic oligonucleotide: CL9
  source 1..34: mol_type = other DNA
gtgactggagttcagacgtgtgctcttccgatct

SEQ ID NO: 2 - DNA, 16 bp, synthetic construct
  misc_feature 1..16: note = Synthetic oligonucleotide: Adapter 2.1
  misc_feature 16: note = ddT at 3' end
  source 1..16: mol_type = other DNA
cgacgctcttccgatc

SEQ ID NO: 3 - DNA, 34 bp, synthetic construct
  misc_feature 1..34: note = Synthetic oligonucleotide: Adapter 2.2
  misc_feature 1: note = 5Phos at 5' end
  misc_feature 30..31: note = Phosphorothioate bond
  misc_feature 31..32: note = Phosphorothioate bond
  misc_feature 32..33: note = Phosphorothioate bond
  misc_feature 33..34: note = Phosphorothioate bond
  source 1..34: mol_type = other DNA
agatcggaagagcgtcgtgtagggaaagagtgta

SEQ ID NO: 4 - DNA, 10 bp, synthetic construct
  misc_feature 1..10: note = Synthetic oligonucleotide: CL78
  misc_feature 1: note = 5Phos at 5' end
  misc_feature 10: note = (iSpC3)10 and 3BioTEG at 3' end
  source 1..10: mol_type = other DNA
agatcggaag